European Patent Application EP 4 474 821 A1, published December 11, 2024. Title: METHODS FOR DIAGNOSING OR MONITORING MUSCULAR GLYCOGENOSIS. Applicant: GENETHON. Application EP. The sequence listing filed with the application follows.

SEQUENCE LISTING (24 sequences)

SEQ ID NO: 1 - protein, 1685 aa, Homo sapiens
MSLPFYQRCHQHYDLSYRNKDVRSTVSHYQREKKRSAVYTQGSTAYSSRSSAAHRRESEAFRRASASSSQQQASQHALSSEVSRKAASAYDYGSSHGLTDSSLLLDDYSSKLSPKPKRAKHSLLSGEEKENLPSDYMVPIFSGRQKHVSGITDTEEERIKEAAAYIAQRNLLASEEGITTSKQSTASKQTTASKQSTASKQSTASKQSTASRQSTASRQSVVSKQATSALQQEETSEKKSRKVVIREKAERLSLRKTLEETETYHAKLNEDHLLHAPEFIIKPRSHTVWEKENVKLHCSIAGWPEPRVTWYKNQVPINVHANPGKYIIESRYGMHTLEINGCDFEDTAQYRASAMNVKGELSAYASVVVKRYKGEFDETRFHAGASTMPLSFGVTPYGYASRFEIHFDDKFDVSFGREGETMSLGCRVVITPEIKHFQPEIQWYRNGVPLSPSKWVQTLWSGERATLTFSHLNKEDEGLYTIRVRMGEYYEQYSAYVFVRDADAEIEGAPAAPLDVKCLEANKDYIIISWKQPAVDGGSPILGYFIDKCEVGTDSWSQCNDTPVKFARFPVTGLIEGRSYIFRVRAVNKMGIGFPSRVSEPVAALDPAEKARLKSRPSAPWTGQIIVTEEEPSEGIVPGPPTDLSVTEATRSYVVLSWKPPGQRGHEGIMYFVEKCEAGTENWQRVNTELPVKSPRFALFDLAEGKSYCFRVRCSNSAGVGEPSEATEVTVVGDKLDIPKAPGKIIPSRNTDTSVVVSWEESKDAKELVGYYIEASVAGSGKWEPCNNNPVKGSRFTCHGLVTGQSYIFRVRAVNAAGLSEYSQDSEAIEVKAAIGGGVSPDVCPALSDEPGGLTASRGRVHEASPPTFQKDALLGSKPNKPSLPSSSQNLGQTEVSKVSETVQEELTPPPQKAAPQGKSKSDPLKKKTDRAPPSPPCDITCLESFRDSMVLGWKQPDKIGGAEITGYYVNYREVIDGVPGKWREANVKAVSEEAYKISNLKENMVYQFQVAAMNMAGLGAPSAVSECFKCEEWTIAVPGPPHSLKCSEVRKDSLVLQWKPPVHSGRTPVTGYFVDLKEAKAKEDQWRGLNEAAIKNVYLKVRGLKEGVSYVFRVRAINQAGVGKPSDLAGPVVAETRPGTKEVVVNVDDDGVISLNFECDKMTPKSEFSWSKDYVSTEDSPRLEVESKGNKTKMTFKDLGMDDLGIYSCDVTDTDGIASSYLIDEEELKRLLALSHEHKFPTVPVKSELAVEILEKGQVRFWMQAEKLSGNAKVNYIFNEKEIFEGPKYKMHIDRNTGIIEMFMEKLQDEDEGTYTFQLQDGKATNHSTVVLVGDVFKKLQKEAEFQRQEWIRKQGPHFVEYLSWEVTGECNVLLKCKVANIKKETHIVWYKDEREISVDEKHDFKDGICTLLITEFSKKDAGIYEVILKDDRGKDKSRLKLVDEAFKELMMEVCKKIALSATDLKIQSTAEGIQLYSFVTYYVEDLKVNWSHNGSAIRYSDRVKTGVTGEQIWLQINEPTPNDKGKYVMELFDGKTGHQKTVDLSGQAYDEAYAEFQRLKQAAIAEKNRARVLGGLPDVVTIQEGKALNLTCNVWGDPPPEVSWLKNEKALASDDHCNLKFEAGRTAYFTINGVSTADSGKYGLVVKNKYGSETSDFTVSVFIPEEEARMAALESLKGGKKAK

SEQ ID NO: 2 - protein, 1667 aa, Mus musculus
MSLPFYQRSHQHYDLSYRNKDLRTTMSHYQQEKKRSAVYTHGSTAYSSRSLAARRQESEAFSQASATSYQQQASQTYSLGASSSSRHSQGSEVSRKTASAYDYGYSHGLTDSSLLLEDYSSKLSPQTKRAKRSLLSGEETGSLPGNYLVPIYSGRQVHISGIRDSEEERIKEAAAYIAQKTLLASEEAIAASKQSTASKQSATSKRTTSTLQREETFEKKSRNIAIREKAEELSLKKTLEETQTYHGKLNEDHLLHAPEFIIKPRSHTVWEKENVKLHCSVAGWPEPRLTWYKNQVPINVHANPGKYIIESRYGMHTLEISKCDFEDTAQYRASAMNVQGELSAYASVVVKRYKGELDESLLRGGVSMPLSFAVTPYGYASKFEIHFDDKFDVSFGREGETMSLGCRVVITPEIKHFQPEVQWYRNGAPVSPSKWVQPHWSGDRATLTFSHLNKEDEGLYTIRVRMGEYYEQYSAYVFVRDADAEIEGAPAAPLDVVSLDANKDYIIISWKQPAVDGGSPILGYFIDKCEVGTDTWSQCNDTPVKFARFPVTGLIEGRSYIFRVRAVNKTGIGLPSRVSEPVAALDPAEKARLKSHPSAPWTGQIIVTEEEPTEGVIPGPPTDLSVTEATRSYVVLSWKPPGQRGHEGIMYFVEKCDVGAENWQRVNTELPVKSPRFALFDLVEGKSYRFRVRCSNSAGVGEPSETTEVTVVGDKLDIPKAPGKIIPSRNTDTSVVVSWEESRDAKELVGYYIEASVVGSGKWEPCNNNPVKGSRFTCHGLTTAQSYIFRVRAVNAAGLSEYSQDSEAIEVKAAIGGGVSPDVWPQLSDTPGGLTDSRGGMNGASPPTSQKDALLGSNPNKPSPPSSPSSRGQKEVSTVSESVQEPLSSPPQEAAPEEEQSQSEPPKKKKDPVAVPSAPYDITCLESFRDSMVLGWKQPDTTGGAEITGYYVNYREVVGEVPGKWREANIKAVSDAAYKISNLKENTLYQFQVSAMNIAGLGAPSTVSECFKCEEWTIAVPGPPHSVKLSEVRKNSLVLQWKPPVYSGRTPVTGYFVDLKEASAKDDQWRGLNEAAIVNKYLRVQGLKEGTSYVFRVRAVNQAGVGKPSDLAGPVVAETRPGTKEVVVSVDDDGVISLNFECDQMTPKSEFVWSKDYVPTEDSPRLEVENKGDKTKMTFKDLGTDDLGTYSCDVTDTDGIASSYLIDEEEMKRLLALSQEHKFPTVPTKSELAVEILEKGQVRFWMQAEKLSSNAKVSYIFNEKEIFEGPKYKMHIDRNTGIIEMFMEKLQDEDEGTYTFQIQDGKATGHSTLVLIGDVYKKLQKEAEFQRQEWIRKQGPHFAEYLSWEVTGECNVLLKCKVANIKKETHIVWYKDEREISVDEKHDFKDGICTLLITEFSKKDAGFYEVILKDDRGKDKSRLKLVDEAFQDLMTEVCKKIALSATDLKIQSTAEGIRLYSFVCYYLDDLKVNWSHNGTGIKYTDRVKSGVTGEQIWLQINEPTPNDKGKYVMELFDGKTGHQKTVDLSGQAFDEAFAEFQRLKQAAIAEKNRARVLGGLPDVVTIQEGKALNLTCNVWGDPPPEVSWLKNEKPLTSDDHCSLKFEAGKTAFFTISGVSTADSGKYGLVVKNKYGSETSDFTVSVFIPEEELRKGAMEPPKGNQKSK

SEQ ID NO: 3 - protein, 1676 aa, Rattus norvegicus
MSLPFYQRSHQHYDLSYRNKDLHTTMSHYQQEKKRSAVYTHGSTAYSSRSSAAHRQESEALRQASAASYQQQASKAYSLGTSSSQHYQGSEVSRKTASSYDYGYSHGLTDSSLLLEDYSSRLSPQTKRAKRSLLSGEETGNLSGNYMVPIYSGRQVHISGIRDSEEERIKEAAAYIAQRTLLESEEAIMASKQSTASKQSTASKQSIASKQSTASKQSTASKQSTASKQATSTFQQEETFERKSRNISIREKAEELSLRKTLEETQAYHGKLNEDHLLHAPEFIIKPRSHTVWEKENVKLHCSVAGWPEPRLTWYKNQVPINVHANPEKYIIESRYGMHTLEISKCDFEDTAQYRASAMNVQGEVSAYASVVVKRYKGELDDSLLRGGVSMPLSFAVTPYGYASKFEIHFDDKFDVSFGREGETMSLGCRVVITPEIKHVQPEVQWYRNGAPVSPSKWVQPHWSGDRATLTFSHLNKEDEGLYTIRVRMGEYYEQYSAYVFVRDADAEIEGAPAAPLDVVSLDANKDYIIISWKQPAVDGGSPILGYFIDKCEVGTDTWSQCNDTPVKFARFPVTGLIEGRSYIFRVRAVNKTGIGLPSRVSEPVAALDPAEKARLKSRPSAPWTGQIIVTEEEPTEGVIPGPPTDLSVTEATRSYVVLSWKPPGQRGHEGIMYFVEKCDVGTENWQRVNTELPVKSPRFALFDLVEGKSYRFRVRCSNSAGVGEPSESTEVTVVGDKLDIPKAPGKIIPSRNTDTSVVVSWEESKDAKELVGYYIESSVVGSGQWEPCNNNPVKGSRFTCHGLTTGQSYIFRVRAVNAAGLSEYSQDSEAIEVKAAIGGGVSPDVWPQLSDTPGGLTDSGGAMSGASPPTSQKDALPSSKPNKPSPPSSPSNRGQKEVSKVNGSVQEELSPPSMEVASKEQSKSGPPEKKKDPVAVPSPPYDITCLESFRDSMVLGWKQPDKTGGAEITGYYVNYREVVGGVPGKWREANIKAVSDAAYKISELKENTVYQFQVSAMNIAGLGAPSAVSECFKCEEWTIAVPGPPHSLKLSEVRKNSLVLQWKPPVYSGRTPVTGYFVDLKEASAKDDQWRGLNEAAIPNKYLRVQGLKEGISYVFRVRAINQAGVGKPSDLAGPVVAETRPGTKEVVVNVDDDGVISLNFECDQMTPKSEFVWSKDYVPSEDSPRLEVESKGNKTKMVFKDLGPDDLGTYSCDVTDTDGIASSYLIDEEEMKRLLALSQEHKFPTVPTKSELAVEILEKGQVRFWMQAEKLSGNAKVNYIFNEKEIFEGPKYKMHIDRNTGIIEMFMEKLQDEDEGTYTFQIQDGKATGHSTLVLIGDVYKKLQKEAEFQRQEWIRKQGPHFAEYLSWEVTGECNVLLKCKVANIKKETHIVWYKDEREISVDEKHDFKDGICTLLITEFSKKDAGFYEVILKDDRGKDKSRLKLVDEAFQDLMTEVCRKIALSATDLKIQSTAEGIRLYSFVCYYLDDLKVNWSHNGTGIKYTDRVKSGVTGEQIWLQINEPTQNDKGKYVMELFDGKTGHQKSVDLSGQAFDEAFAEFQRLNGFITFLPVTLSLQALNLTCNVWGDPTPEVSWLKNEKPLTSDDHCSLKFEAGKTAFFTISGVSTADSGKYGLVVKNKYGSETSDFTVSVFIPEEEARKGASEPPKGNQKSK

SEQ ID NO: 4 - protein, 1465 aa, Homo sapiens
MSLVTVPFYQKRHRHFDQSYRNIQTRYLLDEYASKKRASTQASSQKSLSQRSSSQRASSQTSLGGTICRVCAKRVSTQEDEEQENRSRYQSLVAAYGEAKRQRFLSELAHLEEDVHLARSQARDKLDKYAIQQMMEDKLAWERHTFEERISRAPEILVRLRSHTVWERMSVKLCFTVQGFPTPVVQWYKDGSLICQAAEPGKYRIESNYGVHTLEINRADFDDTATYSAVATNAHGQVSTNAAVVVRRFRGDEEPFRSVGLPIGLPLSSMIPYTHFDVQFLEKFGVTFRREGETVTLKCTMLVTPDLKRVQPRAEWYRDDVLLKESKWTKMFFGEGQASLSFSHLHKDDEGLYTLRIVSRGGVSDHSAFLFVRDADPLVTGAPGAPMDLQCHDANRDYVIVTWKPPNTTTESPVMGYFVDRCEVGTNNWVQCNDAPVKICKYPVTGLFEGRSYIFRVRAVNSAGISRPSRVSDAVAALDPLDLRRLQAVHLEGEKEIAIYQDDLEGDAQVPGPPTGVHASEISRNYVVLSWEPPTPRGKDPLMYFIEKSVVGSGSWQRVNAQTAVRSPRYAVFDLMEGKSYVFRVLSANRHGLSEPSEITSPIQAQDVTVVPSAPGRVLASRNTKTSVVVQWDRPKHEEDLLGYYVDCCVAGTNLWEPCNHKPIGYNRFVVHGLTTGEQYIFRVKAVNAVGMSENSQESDVIKVQAALTVPSHPYGITLLNCDGHSMTLGWKVPKFSGGSPILGYYLDKREVHHKNWHEVNSSPSKPTILTVDGLTEGSLYEFKIAAVNLAGIGEPSDPSEHFKCEAWTMPEPGPAYDLTFCEVRDTSLVMLWKAPVYSGSSPVSGYFVDFREEDAGEWITVNQTTTANRYLKVSDLQQGKTYVFRVRAVNANGVGKPSDTSEPVLVEARPGTKEISAGVDEQGNIYLGFDCQEMTDASQFTWCKSYEEISDDERFKIETVGDHSKLYLKNPDKEDLGTYSVSVSDTDGVSSSFVLDPEELERLMALSNEIKNPTIPLKSELAYEIFDKGRVRFWLQAEHLSPDASYRFIINDREVSDSEIHRIKCDKATGIIEMVMDRFSIENEGTYTVQIHDGKAKSQSSLVLIGDAFKTVLEEAEFQRKEFLRKQGPHFAEYLHWDVTEECEVRLVCKVANTKKETVFKWLKDDVLYETETLPNLERGICELLIPKLSKKDHGEYKATLKDDRGQDVSILEIAGKVYDDMILAMSRVCGKSASPLKVLCTPEGIRLQCFMKYFTDEMKVNWCHKDAKISSSEHMRIGGSEEMAWLQICEPTEKDKGKYTFEIFDGKDNHQRSLDLSGQAFDEAFAEFQQFKAAAFAEKNRGRLIGGLPDVVTIMEGKTLNLTCTVFGNPDPEVIWFKNDQDIQLSEHFSVKVEQAKYVSMTIKGVTSEDSGKYSINIKNKYGGEKIDVTVSVYKHGEKIPDMAPPQQAKPKLIPASASAAGQ

SEQ ID NO: 5 - protein, 1463 aa, Mus musculus
MSLVAVPFYQKRHKHFDQSYRNIQTRYLLDQYALKKQATTQSSSQRSLTERSSSKRASSQSSAGAMTCRLCAKRVSASEEEEVENENRYRSQAASYGEAKRQRFLSELAQLEENVHLARSQARDKLDKYFMEQTVEDNLAWERHSFEYRMSRAPEILVRLRSHTIWERMSVRLCFTVQGFPTPVVQWYKDGSLICQAGEPGKYRIESRYGVHTLEINRANFEDTATYSAVATNSHGQVSTNAAVVVRRYRGEEEPFHSVGLPIGLPLSSVIPYTHFDVQFLEKFGVTFRREGETVTLKCTLLVTPDLKRVQPRAEWYRDDVLLKESKWTKMFFGEGQASLSFSHLNKDDEGLYTLRIVSRGGVSDHSAFMFVRDADPLVTGAPGAPMDLQCHDANRDYVIVTWKPPNTTTESPVIGYFIDKCEVGTNNWVQCNDAPVKICKYPVTGLFEGRSYVFRVRAVNNAGISRPSRISDAVAALDPVDLRRLQAIHLEGEKEIVIYQDDLEGDVQIPGPPTNVQASEVSRNYVVLSWDPPSPRGKDPLMYFIEKSAVGSGSWQRVNAQTAVRSPRYAVFDLAEGKSYVFRVLSANKHGLSDPSEITPPIQAQDMIVVPSAPGRVLASRNTKTSVVVQWDRPKHEEDLLGYYVDCCVAGTNMWEPCNHKPIGYNRFVVHGLTTGEQYIFRVKAVNAVGTSENSQESEVIKVQAALTVPSHPYGITLLNCDGHSMTLGWKVPKFSGGSAIIGYYLDKREVHHKNWHEVNSSPVKERILTVEGLTEGSLYEFKIAATNLAGIGQPSDPSEHFKCEAWTDPEPGPAYDLTFCEVRDTSLVILWKAPVYSGSSPVSGYFVDFKEEDSGEWKTTSEAATPNRYLKVCDLQQGKTYVFRIRAVNASGPGKPSDTSEPVLVEARPGTKEISAGVDEEGNIYLGFDCQEMTDASQFTWCKAYEEIADEERFEVHTEGDHSKLYFKNPDKEDLGTYSVSVSDTDGVSSSFVLDEEELERLMALSNEIKNPTIPLKSELAYEIFDKGQVRFWLQAEHLSPDASFRFIINDREVSDSDTHRIKCDRSTGMIEMVMDRFTIENEGTYTVQIQDGKAKNQSSLVLIGDAFKAVLEEAEFQRKEFLRKQGPHFAEYLHWDVTEECEVRLVCKVANTKRETVFKWLKDDVLYETETPPDLEKGVCELLIPKLSKKDHGEYKATLKDDRGQDVSVLEVGGKVYEDMILAMSRVCGASASPLKVLCTPEGIRLQCFMKYFTEEMKVSWYHKEAKISSSEHMRIGGSEEMAWLQICEPTEKDKGKYTFEIFDGKDSHQRSLDLSGQAFDEAYAEFQQLKAAAFAEKNRGKVIGGLPDVVTIMEGKTLNLTCTVFGNPDPEVVWFKNDKDIELSEHFLVKMEQSKYVSLTIQGVTAEDSGKYSINVKNKYGGEKIDVTVSVYKHGEKIPDISPPQQAKPKLIPASTSSD

SEQ ID NO: 6 - protein, 1541 aa, Rattus norvegicus
MGLGEAALCLNIAPPLAINGGKHGALQGEISSAVLGQCLGNSSTALFVSAGFFPLECERQRAQDRLLKIISLSGISKMSLVVVPFYQKRHKHFDQSYRNIQTRYLLDRYASKKQASSQSSSQRSLTERSSSKRASSQSSAEGMTCRLCAKRMSASEEEEVENENRYRSLAASYGEAKRQRFLSELAQLEENVQLARTQARNKLDKYFLEQTVADNLALERSSFEDRLSRAPEILVRLRSHTIWERMSVRLCFTVQGFPTPVVQWYKDGSLICQAGEPGKYRIESRYGVHTLEINRADFEDTATYSAVATNPHGQVSTNAAVVVRRYRGDEEPYHSVGLPIGLPLSSVIPYTHFDVQFLEKFGVTFRREGETVTLKCTLLVTPDLKRVQPRAEWYRDDVLLKESKWTKMFFGEGQASLSFSHLNKDDEGLYTLRIVSRGGVSDHSAFMFVRDADPLVTGAPGAPMDLQCHDANRDYVIVTWKPPNTTTESPVIGYFIDKCEVGTNNWVQCNDAPVKICKYPVTGLFEGRSYVFRVRAVNNAGISRPSRISDAVAALDPVDLRRLQAIHLEGEKEIVIYQDDLEGDVQIPGPPTNVQASEVSRNYVVLSWDPPSPRGKEPLMYFIEKSAVGSGSWQRVNAQTAVRSPRYAVFDLAEGKSYVFRVLSANKHGLSDPSEITPPIQAQDMIVVPSAPGRVLASRNTKTSVVVQWDRPKHEEDLLGYYVDCCVAGTNMWEPCNHKPIGYNRFVVHGLTTGEQYIFRVKAVNAVGTSENSQESEVIKVQAALTVPSHPYGITLLNCDGHSMTLGWKVPKFSGGSAIIGYYLDKREVHHKNWHEINSSPVKERILTVEGLTEGSLYEFKIAATNLAGIGQPSDPSEHFKCEAWTAPEPGPAYDLTFCEVRDTSLVILWKAPVYSGSSPVSGYFVDFKEEDSGEWKTTSEAATPNRYLKVCDLHQGKTYVFRVRAVNASGPGKPSDTSEPVLVEARPGTKEISAGVDEEGNIYLGFDCQEMTDASQFTWCKAYEEIADEERFEVHTEGDHSKLYFKNPDKIDIGTYSVSVSDTDGVSSSFVLDEEELERLMALSNEIKNPTIPLKSELAYEIFDKGQVRFWLQAEHLSPDANFRFIINDREVSDSETHRIKCDRSTGMIEMVMDRFTIENEGTYTVQIQDGKAKNQSSLVLIGDAFRAVLEEAEFQRKEFLRKQGPHFAEYLHWDVTEECEVRLICKVANTKRETVFKWLKDDVLYETETPPPDLEKGICELLIPKLSKKDHGEYKATLKDDRGQDVSVLEVAGKVYEDMILAMSRVCGASASPLKVLCTPEGIRLQCFMKYFTEEMKVSWYHKEAKISSSEHMRIGGSEEMAWLQICEPTEKDKGKYTFEIFDGKDNHQRSLDLSGQAFDEAYAEFQQLKAAAFAEKNRGKVIGGLPDVVTIMEGKTLNLTCTVFGNPDPEVVWFKNDKDIELSEHFSVKVEQSKYVSLTIKGVTAEDSGKYSINVKNKYGGEKIDVTVSVYKHGEKIPDISAPQQAKPKLIPASTSAD

SEQ ID NO: 7 - protein, 1437 aa, Homo sapiens
MTLPHSLGGAGDPRPPQAMEVHRLEHRQEEEQKEERQHSLRMGSSVRRRTFRSSEEEHEFSAADYALAAALALTASSELSWEAQLRRQTSAVELEERGQKRVGFGNDWERTEIAFLQTHRLLRQRRDWKTLRRRTEEKVQEAKELRELCYGRGPWFWIPLRSHAVWEHTTVLLTCTVQASPPPQVTWYKNDTRIDPRLFRAGKYRITNNYGLLSLEIRRCAIEDSATYTVRVKNAHGQASSFAKVLVRTYLGKDAGFDSEIFKRSTFGPSVEFTSVLKPVFAREKEPFSLSCLFSEDVLDAESIQWFRDGSLLRSSRRRKILYTDRQASLKVSCTYKEDEGLYMVRVPSPFGPREQSTYVLVRDAEAENPGAPGSPLNVRCLDVNRDCLILTWAPPSDTRGNPITAYTIERCQGESGEWIACHEAPGGTCRCPIQGLVEGQSYRFRVRAISRVGSSVPSKASELVVMGDHDAARRKTEIPFDLGNKITISTDAFEDTVTIPSPPTNVHASEIREAYVVLAWEEPSPRDRAPLTYSLEKSVIGSGTWEAISSESPVRSPRFAVLDLEKKKSYVFRVRAMNQYGLSDPSEPSEPIALRGPPATLPPPAQVQAFRDTQTSVSLTWDPVKDPELLGYYIYSRKVGTSEWQTVNNKPIQGTRFTVPGLRTGKEYEFCVRSVSEAGVGESSAATEPIRVKQALATPSAPYGFALLNCGKNEMVIGWKPPKRRGGGKILGYFLDQHDSEELDWHAVNQQPIPTRVCKVSDLHEGHFYEFRARAANWAGVGELSAPSSLFECKEWTMPQPGPPYDVRASEVRATSLVLQWEPPLYMGAGPVTGYHVSFQEEGSEQWKPVTPGPISGTHLRVSDLQPGKSYVFQVQAMNSAGLGQPSMPTDPVLLEDKPGAHEIEVGVDEEGFIYLAFEAPEAPDSSEFQWSKDYKGPLDPQRVKIEDKVNKSKVILKEPGLEDLGTYSVIVTDADEDISASHTLTEEELEKLKKLSHEIRNPVIKLISGWNIDILERGEVRLWLEVEKLSPAAELHLIFNNKEIFSSPNRKINFDREKGLVEVIIQNLSEEDKGSYTAQLQDGKAKNQITLTLVDDDFDKLLRKADAKRRDWKRKQGPYFERPLQWKVTEDCQVQLTCKVTNTKKETRFQWFFQRAEMPDGQYDPETGTGLLCIEELSKKDKGIYRAMVSDDRGEDDTILDLTGDALDAIFTELGRIGALSATPLKIQGTEEGIRIFSKVKYYNVEYMKTTWFHKDKRLESGDRIRTGTTLDEIWLHILDPKDSDKGKYTLEIAAGKEVRQLSTDLSGQAFEDAMAEHQRLKTLAIIEKNRAKVVRGLPDVATIMEDKTLCLTCIVSGDPTPEISWLKNDQPVTFLDRYRMEVRGTEVTITIEKVNSEDSGRYGVFVKNKYGSETGQVTISVFKHGDEPKELKSM

SEQ ID NO: 8 - protein, 1439 aa, Mus musculus
MTLPHSPGSAGEPQASQTVQVHRLEHRQEEEQKEERQHSLQMGSSVQRRTYRSSEEEQQFSSEDYALAAALALTASSELSWEAKLRRQTTTVELEERGQRRVGFGNDLERMELAFLRTQRLLRQRRDWKALRQRTEEKVREAKELIELCSGRGPWFWIPLRSHAVWEHTTVLLTCTVQGSPPFQVTWYKNDIRIDPRLFPAGKYRITNNYGLLTLEIMRCTVEDSATYTVLVKNAYGQASSFAKVLIRNYLGKDAGFDSEIFKRSMFGPSAEFTSVLKPIFAQEKEPFSLTCLFSDDVLEAEQRIQWYRDGRLLRSSTRRQILYADRQASVKVSCAYKEDEGFYTIRVSSPFGPQEQSAYVFIRDAAAEKPGAPGSPLNVRCLNVHRDCLTLTWVPPSDTRGSTITGYSIEMCQGDSEEWMPCLKAPGGTCRCPIQGLVEGQSYQFRVRAISKAGTSLPSKASEAVVTGDYDAVHKSTEIPYDLGSKITISKNDFEDAVTIPSAPTNVHASEIREAYAVLSWEEPRPRGRAPLTYTLEKSVIGSGTWEAISTETPIKSPRFALLDLEKGKSYVFRVRALNQYGMSDPSEPSEPVALKGKPATLPPPAQVQAFRNTQTSVSLAWEPVDGGSELLGYYIYSREAGASEWQTVNNKPIQDTKFTVPGLRTGKEYDFCIRSVSEAGVGESSAATQPVRVKQALATPSAPYDFALLNCGKNEMVIGWKPPKRRGGGKILGYFMDQHDSVESDWHPVNRQPIPSRVCKVTNLHEGHFYEFRARAVNWAGIGELSAPSSLFECKEWTMPEPGPPYDVRVSEVQATSVMLQWEPPLYIGAGPVTGYHVSFQEKGSEEWKPVTPDATSDTHLRVSDLQPGKQYMFRVQAMNSAGLGQPSVPTDPVLLEDKPDAQEIEVGVDDEGQIYLAFEAPEAPDFPEFQWSKDYQGPPDPQRVEVEDEISKSKVILKEPDLQDLGIYSVVVPDADEDTSASHTLTEEELNKLKKLSHEIRNPVIKLISGWNVEILEQGEVRLWLEVEKLSPAAELHLIFNEKEIFSSPNRKINFDREKGLVEVIIQQLSEDDKGSYTAQLQDGKAKNQITLALVDDEFDKLLRKADAKRRDWKRKQGPYFQEPLTWKVTDDCQVLLSCKVTNTKKESRFQWFFQKKEAPHGQYNPPTGDGSLSIEGFSKENQGVYRAVVSDERGEDDTVLDLTGEALDAVLTELGRIGALSATPLKIQGTEEGIRLFSKVKYYNVDYMKTAWFHKDKRLESGDRVRAGTTLDEIWLHILDPKDSDKGKYTLEITAGKEVRQLSADLSGQAFDDALAEHQRLKALAVIEKNRAKVVRGLPDVATIMEDKTLCLTCVISGDPSPEISWLKNDQPISFFDRYHMEVKGTEVTVTIDKVTSEDSGRYGIFVKNKYGSETGQVTISVFKHGEEPKELKKK

SEQ ID NO: 9 - protein, 1438 aa, Rattus norvegicus
MTLPHSPGSAGEPQASQTVQVHRLEHKHEEEQKEEREHSLRMGSSVQRRTYRSSEEEQQFSPEDYALAAALALTASSELSWEAKLRRQTTRVELEERGQKRIGFGNDLERMEMAFLRTQRLLRQRRDWKALRQRTEQKVLEAKELIELCSGRGPWFWIPLRSHAVWEYTTVLLTCTIQGSFPFQVTWYKDDIQIDPRLFPAGKYRITNNYGLLTLEIRRCTVEDSATYTVLVKNAFGQASSFAKVLIRTYLGKDAGFDSEIFKRSMFGPTVEFTSVLKPIFAQEKEPFSLTCLFSDDVLEAEERIQWFRDGRLLRSSTRRQILYADRQASVKVSCAYKEDEGFYTIRVSSPFGPQEQSAYVFIRDAAAEKPGAPGSPLNVRCLNVHRDCLTLTWVPPSDTRGSTITGYSIELCQGDSEEWVPCLKTPGGTCRCPIQGLIEGQSYRFRVRAISKAGTSLPSKASAAVVMGDYDTVQKKTEIPFDLGRKITISKNDFEDAVTIPSAPTNVHASEIRDTYAVLSWEEPHPRGRAPLTYTLEKSVIGSGTWEAISSETPIKSPRFALLDLEKGKSYVFRVRALNQYGMSDPSEPSEPITLKGKPATLPPPAQVQSFRNTQTSVSLTWEPVDGGSELLGYYIYSREAGASEWQTVNNKPIQDTKFTVPGLRTGKEYEFCIRSVSEAGVGESSAVTQPIRVKQALATPSAPYDFALLNCGKNEMVIGWKPPKRRGGGKILGYYVDQHDSEELDWHPVSHQPNPSRVCKVTNLHEGHFYEFRARAMNWAGIGELSAPSSLFECKEWTMPEPGPPYDVRASEIQATSVMLQWEPPLYIGAGPVTGYRVSFQEIGSEEWKPVTPDATSDTHLRVSDLQPGKQYMFRVQAMNSAGLGQPSVPTDPVLLEDKPDAHEIEVGVDEEGQIYLAFEAPEAPDFPEFQWSKDYKGPPDPQRVEVKDEINKSKVILKEPDLQDLGVYSVVVTDADEDTSASHTLTEEELNKLKKLSHEIRNPVIKLISGWNVDILEQGEVRLWLEVEKLSPAAELHLIFNEKEIFSSPNRKINFDREKGLVEVIIQQLSEDDKGSYTAQLQDGKAKNQITLALVDDDFDKLLRKADAKRRDWKRKQGPYFQDPLTWKVTEDCQVLLTCKVTNTKKETRFQWLFQKKEAPRGQYSPQTGDGSLCIEEFSKEDQGLYRAVVSDERGEDDTVLDLTGEALDAVLTELGRISALSATPLKIQGTEEGIRLFSKVKYYNVDYMKTAWFHKDKRLESGDRVRAGTTLDEIWLHILDPKDSDKGKYTLEITAGKEVCQLSADLSGQAFDDALAEHQRLKALAVIEKNRAKVVRGLPDVATIMEDKTLCLTCVISGDPSPEISWLKNDQPVSFLDRYHMEVKGTEVTITIDKVTSEDSGRYGIFVKNKYGSETGQVTISVFKHGEEPKELKK

SEQ ID NO: 10 - protein, 9 aa, synthetic construct
EQSTYVLVR

SEQ ID NO: 11 - protein, 17 aa, synthetic construct
DAEAENPGAPGSPLNVR

SEQ ID NO: 12 - protein, 14 aa, synthetic construct
ASELVVMGDHDAAR

SEQ ID NO: 13 - protein, 18 aa, synthetic construct
SVIGSGTWEAISSESPVR

SEQ ID NO: 14 - protein, 8 aa, synthetic construct
FAVLDLEK

SEQ ID NO: 15 - protein, 20 aa, synthetic construct
AMNQYGLSDPSEPSEPIALR

SEQ ID NO: 16 - protein, 18 aa, synthetic construct
VGTSEWQTVNNKPIQGTR

SEQ ID NO: 17 - protein, 19 aa, synthetic construct
QALATPSAPYGFALLNCGK

SEQ ID NO: 18 - protein, 13 aa, synthetic construct
VSDLHEGHFYEFR

SEQ ID NO: 19 - protein, 20 aa, synthetic construct
AANWAGVGELSAPSSLFECK

SEQ ID NO: 20 - protein, 12 aa, synthetic construct
LISGWNIDILER

SEQ ID NO: 21 - protein, 11 aa, synthetic construct
GSYTAQLQDGK

SEQ ID NO: 22 - protein, 12 aa, synthetic construct
VTEDCQVQLTCK

SEQ ID NO: 23 - protein, 10 aa, synthetic construct
IGALSATPLK

SEQ ID NO: 24 - protein, 20 aa, synthetic construct
QLSTDLSGQAFEDAMAEHQR